European Patent Specification EP 3 262 178 B1, published February 22, 2023. Title: FLAVIVIRUS REPLICONS. Applicant: NOVARTIS AG. Application EP 15157068.6. The sequence listing filed with the application follows.

SEQUENCE LISTING (27 sequences)

SEQ ID NO: 1 - DNA, 8839 bp, West Nile virus
agtagttcgcctgtgtgagctgacaaacttagtagtgtttgtgaggattaacaacaattaacacagtgcgagctgtttcttagcacgaagatctcgatgtctaagaaaccaggagggcccggcaagagccgggctgtcaatatgctaaaacgcggaatgccccgcgtgttgtccttgattggacttaagatgggcatcaatgctcgtgataggtccatagctctcacgtttctcgcagttggaggagttctgctcttcctctccgtgaacgtgcacgctgacactgggtgtgccatagacatcagccggcaagagctgagatgtggaagtggagtgttcatacacaatgatgtggaggcttggatggaccgatacaagtattaccctgaaacgccacaaggcctagccaagatcattcagaaagctcataaggaaggagtgtgcggtctacgatcagtttccagactggagcatcaaatgtgggaagcagtgaaggacgagctgaacactcttttgaaggagaatggtgtggaccttagtgtcgtggttgagaaacaggagggaatgtacaagtcagcacctaaacgcctcaccgccaccacggaaaaattggaaattggctggaaggcctggggaaagagtattttatttgcaccagaactcgccaacaacacctttgtggttgatggtccggagaccaaggaatgtccgactcagaatcgcgcttggaatagcttagaagtggaggattttggatttggtctcaccagcactcggatgttcctgaaggtcagagagagcaacacaactgaatgtgactcgaagatcattggaacggctgtcaagaacaacttggcgatccacagtgacctgtcctattggattgaaagcaggctcaatgatacgtggaagcttgaaagggcagttctgggtgaagtcaaatcatgtacgtggcctgagacgcataccttgtggggcgatggaatccttgagagtgacttgataataccagtcacactggcgggaccacgaagcaatcacaatcggagacctgggtacaagacacaaaaccagggcccatgggacgaaggccgggtagagattgacttcgattactgcccaggaactacggtcaccctgagtgagagctgcggacaccgtggacctgccactcgcaccaccacagagagcggaaagttgataacagattggtgctgcaggagctgcaccttaccaccactgcgctaccaaactgacagcggctgttggtatggtatggagatcagaccacagagacatgatgaaaagaccctcgtgcagtcacaagtgaatgcttataatgctgatatgattgacccttttcagttgggccttctggtcgtgttcttggccacccaggaggtccttcgcaagaggtggacagccaagatcagcatgccagctatactgattgctctgctagtcctggtgtttgggggcattacttacactgatgtgttacgctatgtcatcttggtgggggcagctttcgcagaatctaattcgggaggagacgtggtacacttggcgctcatggcgaccttcaagatacaaccagtgtttatggtggcatcgtttctcaaagcgagatggaccaaccaggagaacattttgttgatgttggcggctgttttctttcaaatggcttatcacgatgcccgccaaattctgctctgggagatccctgatgtgttgaattcactggcggtagcttggatgatactgagagccataacattcacaacgacatcaaacgtggttgttccgctgctagccctgctaacacccgggctgagatgcttgaatctggatgtgtacaggatactgctgttgatggtcggaataggcagcttgatcagggagaagaggagtgcagctgcaaaaaagaaaggagcaagtctgctatgcttggctctagcctcaacaggacttttcaaccccatgatccttgctgctggactgattacatgtgatcccaaccgtaaacgcggatggcccgcaactgaagtgatgacagctgtcggcctgatgtttgccatcgtcggagggctggcagagcttgacattgactccatggccattccaatgactatcgcggggctcatgtttgctgctttcgtgatttctgggaaatcaacagatatgtggattgagagaacggcggacatttcctgggaaagtgatgcagaaattacaggctcgagcgaaagagttgatgtgcggcttgatgatgatggaaacttccagctcatgaatgatccaggagcaccttggaagatatggatgctcagaatggtctgtctcgcgattagtgcgtacaccccctgggcaatcttgccctcagtagttggattttggataactctccaatacacaaagagaggaggcgtgttgtgggacactccctcaccaaaggagtacaaaaagggggacacgaccaccggcgtctacaggatcatgactcgtgggctgctcggcagttatcaagcaggagcgggcgtgatggttgaaggtgttttccacaccctttggcatacaacaaaaggagccgctttgatgagcggagagggccgcctggacccatactggggcagtgtcaaggaggatcgactttgttacggaggaccctggaaattgcagcacaagtggaacgggcaggatgaggtgcagatgattgtggtggaacctggcaagaacgttaagaacgtccagacgaaaccaggggtgttcaaaacacctgaaggagaaatcggggccgtgactttggacttccccactggaacatcaggctcaccaatagtggacaaaaacggtgatgtgattgggctttatggcaatggagtcataatgcccaacggctcatacataagcgcgatagtgcagggtgaaaggatggatgagccaatcccagccggattcgaacctgagatgctgaggaaaaaacagatcactgtactggatctccatcccggcgccggtaaaacaaggaggattctgccacagatcatcaaagaggccataaacagaagactgagaacagccgtgctagcaccaaccagggttgtggctgctgagatggctgaagcactgagaggactgcccatccggtaccagacatccgcagtgcccagagaacataatggaaatgagattgttgatgtcatgtgtcatgctaccctcacccacaggctgatgtctcctcacagggtgccgaactacaacctgttcgtgatggatgaggctcatttcaccgacccagctagcattgcagcaagaggttacatttccacaaaggtcgagctaggggaggcggcggcaatattcatgacagccaccccaccaggcacttcagatccattcccagagtccaattcaccaatttccgacttacagactgagatcccggatcgagcttggaactctggatacgaatggatcacagaatacaccgggaagacggtttggtttgtgcctagtgtcaagatggggaatgagattgccctttgcctacaacgtgctggaaagaaagtagtccaattgaacagaaagtcgtacgagacggagtacccaaaatgtaagaacgatgattgggactttgttatcacaacagacatatctgaaatgggggctaactttaaggcgagcagggtgattgacagccggaagagtgtgaaaccaaccatcataacagaaggagaagggagagtgatcctgggagaaccatctgcagtgacagcagctagtgccgcccagagacgtggacgtatcggtagaaatccgtcgcaagttggtgatgagtactgttatggggggcacacgaatgaagacgactcgaacttcgcccattggactgaggcacgaatcatgctggacaacatcaacatgccaaacggactgatcgctcaattctaccaaccagagcgtgagaaggtatataccatggatggggaataccggctcagaggagaagagagaaaaaactttctggaactgttgaggactgcagatctgccagtttggctggcttacaaggttgcagcggctggagtgtcataccacgaccggaggtggtgctttgatggtcctaggacaaacacaattttagaagacaacaacgaagtggaagtcatcacgaagcttggtgaaaggaagattctgaggccgcgctggattgacgccagggtgtactcggatcaccaggcactaaaggcgttcaaggacttcgcctcgggaaaacgttctcagatagggctcattgaggttctgggaaagatgcctgagcacttcatggggaagacatgggaagcacttgacaccatgtacgttgtggccactgcagagaaaggaggaagagctcacagaatggccctggaggaactgccagatgctcttcagacaattgccttgattgccttattgagtgtgatgaccatgggagtattcttcctcctcatgcagcggaagggcattggaaagataggtttgggaggcgctgtcttgggagtcgcgacctttttctgttggatggctgaagttccaggaacgaagatcgccggaatgttgctgctctcccttctcttgatgattgtgctaattcctgagccagagaagcaacgttcgcagacagacaaccagctagccgtgttcctgatttgtgtcatgacccttgtgagcgcagtggcagccaacgagatgggttggctagataagaccaagagtgacataagcagtttgtttgggcaaagaattgaggtcaaggagaatttcagcatgggagagtttcttctggacttgaggccggcaacagcctggtcactgtacgctgtgacaacagcggtcctcactccactgctaaagcatttgatcacgtcagattacatcaacacctcattgacctcaataaacgttcaggcaagtgcactattcacactcgcgcgaggcttccccttcgtcgatgttggagtgtcggctctcctgctagcagccggatgctggggacaagtcaccctcaccgttacggtaacagcggcaacactccttttttgccactatgcctacatggttcccggttggcaagctgaggcaatgcgctcagcccagcggcggacagcggccggaatcatgaagaacgctgtagtggatggcatcgtggccacggacgtcccagaattagagcgcaccacacccatcatgcagaagaaagttggacagatcatgctgatcttggtgtctctagctgcagtagtagtgaacccgtctgtgaagacagtacgagaagccggaattttgatcacggccgcagcggtgacgctttgggagaatggagcaagctctgtttggaacgcaacaactgccatcggactctgccacatcatgcgtgggggttggttgtcatgtctatccataacatggacactcataaagaacatggaaaaaccaggactaaaaagaggtggggcaaaaggacgcaccttgggagaggtttggaaagaaagactcaaccagatgacaaaagaagagttcactaggtaccgcaaagaggccatcatcgaagtcgatcgctcagcagcaaaacacgccaggaaagaaggcaatgtcactggagggcatccagtctctaggggcacagcaaaactgagatggctggtcgaacggaggtttctcgaaccggtcggaaaagtgattgaccttggatgtggaagaggcggttggtgttactatatggcaacccaaaaaagagtccaagaagtcagagggtacacaaagggcggtcccggacatgaagagccccaactagtgcaaagttatggatggaacattgtcaccatgaagagtggggtggatgtgttctacagaccttctgagtgttgtgacaccctcctttgtgacatcggagagtcctcgtcaagtgctgaggttgaagagcataggacgattcgggtccttgaaatggttgaggactggctgcaccgagggccaagggaattttgcgtgaaggtgctctgcccctacatgccgaaagtcatagagaagatggagctgctccaacgccggtatggggggggactggtcagaaacccactctcacggaattccacgcacgagatgtattgggtgagtcgagcttcaggcaatgtggtacattcagtgaatatgaccagccaggtgctcctaggaagaatggaaaaaaggacctggaagggaccccaatacgaggaagatgtaaacttgggaagtggaaccagggcggtgggaaaacccctgctcaactcagacaccagtaaaatcaagaacaggattgaacgactcaggcgtgagtacagttcgacgtggcaccacgatgagaaccacccatatagaacctggaactatcacggcagttatgatgtgaagcccacaggctccgccagttcgctggtcaatggagtggtcaggctcctctcaaaaccatgggacaccatcacgaatgttaccaccatggccatgactgacactactcccttcgggcagcagcgagtgttcaaagagaaggtggacacgaaagctcctgaaccgccagaaggagtgaagtacgtgctcaacgagaccaccaactggttgtgggcgtttttggccagagaaaaacgtcccagaatgtgctctcgagaggaattcataagaaaggtcaacagcaatgcagctttgggtgccatgtttgaagagcagaatcaatggaggagcgccagagaggcagttgaagatccaaaattttgggagatggtggatgaggagcgcgaggcacatctgcggggggaatgtcacacttgcatttacaacatgatgggaaagagagagaaaaaacccggagagttcggaaaggccaagggaagcagagccatttggttcatgtggctcggagctcgctttctggagttcgaggctctgggttttctcaatgaagaccactggcttggaagaaagaactcaggaggaggtgtcgagggcttgggcctccaaaaactgggttacatcctgcgtgaagttggcacccggcctgggggcaagatctatgctgatgacacagctggctgggacacccgcatcacgagagctgacttggaaaatgaagctaaggtgcttgagctgcttgatggggaacatcggcgtcttgccagggccatcattgagctcacctatcgtcacaaagttgtgaaagtgatgcgcccggctgctgatggaagaaccgtcatggatgttatctccagagaagatcagagggggagtggacaagttgtcacctacgccctaaacactttcaccaacctggccgtccagctggtgaggatgatggaaggggaaggagtgattggcccagatgatgtggagaaactcacaaaagggaaaggacccaaagtcaggacctggctgtttgagaatggggaagaaagactcagccgcatggctgtcagtggagatgactgtgtggtaaagcccctggacgatcgctttgccacctcgctccacttcctcaatgctatgtcaaaggttcgcaaagacatccaagagtggaaaccgtcaactggatggtatgattggcagcaggttccattttgctcaaaccatttcactgaattgatcatgaaagatggaagaacactggtggttccatgccgaggacaggatgaattggtaggcagagctcgcatatctccaggggccggatggaacgtccgcgacactgcttgtctggctaagtcttatgcccagatgtggctgcttctgtacttccacagaagagacctgcggctcatggccaacgccatttgctccgctgtccctgtgaattgggtccctaccggaagaaccacgtggtccatccatgcaggaggagagtggatgacaacagaggacatgttggaggtctggaaccgtgtttggatagaggagaatgaatggatggaagacaaaaccccagtggagaaatggagtgacgtcccatattcaggaaaacgagaggacatctggtgtggcagcctgattggcacaagagcccgagccacgtgggcagaaaacatccaggtggctatcaaccaagtcagagcaatcatcggagatgagaagtatgtggattacatgagttcactaaagagatatgaagacacaactttggttgaggacacagtactgtagatatttaatcaattgtaaatagacaatataagtatgcataaaagtgtagttttatagtagtatttagtggtgttagtgtaaatagttaagaaaattttgaggagaaagtcaggccgggaagttcccgccaccggaagttgagtagacggtgctgcctgcgactcaaccccaggaggactgggtgaacaaagccgcgaagtgatccatgtaagccctcagaaccgtctcggaaggaggaccccacatgttgtaacttcaaagcccaatgtcagaccacgctacggcgtgctactctgcggagagtgcagtctgcgatagtgccccaggaggactgggttaacaaaggcaaaccaacgccccacgcggccctagccccggtaatggcgttaaccagggcgaaaggactagaggttagaggagaccccgcggtttaaagtgcacggcccagcctggctgaagctgtaggtcaggggaaggactagaggttagtggagaccccgtgccacaaaacaccacaacaaaacagcatattgacacctgggatagactaggagatcttctgctctgcacaaccagccacacggcacagtgcgccgacaatggtggctggtggtgcgagaacacaggatct

SEQ ID NO: 2 - protein, 2703 aa, West Nile virus
MSKKPGGPGKSRAVNMLKRGMPRVLSLIGLKMGINARDRSIALTFLAVGGVLLFLSVNVHADTGCAIDISRQELRCGSGVFIHNDVEAWMDRYKYYPETPQGLAKIIQKAHKEGVCGLRSVSRLEHQMWEAVKDELNTLLKENGVDLSVVVEKQEGMYKSAPKRLTATTEKLEIGWKAWGKSILFAPELANNTFVVDGPETKECPTQNRAWNSLEVEDFGFGLTSTRMFLKVRESNTTECDSKIIGTAVKNNLAIHSDLSYWIESRLNDTWKLERAVLGEVKSCTWPETHTLWGDGILESDLIIPVTLAGPRSNHNRRPGYKTQNQGPWDEGRVEIDFDYCPGTTVTLSESCGHRGPATRTTTESGKLITDWCCRSCTLPPLRYQTDSGCWYGMEIRPQRHDEKTLVQSQVNAYNADMIDPFQLGLLVVFLATQEVLRKRWTAKISMPAILIALLVLVFGGITYTDVLRYVILVGAAFAESNSGGDVVHLALMATFKIQPVFMVASFLKARWTNQENILLMLAAVFFQMAYHDARQILLWEIPDVLNSLAVAWMILRAITFTTTSNVVVPLLALLTPGLRCLNLDVYRILLLMVGIGSLIREKRSAAAKKKGASLLCLALASTGLFNPMILAAGLITCDPNRKRGWPATEVMTAVGLMFAIVGGLAELDIDSMAIPMTIAGLMFAAFVISGKSTDMWIERTADISWESDAEITGSSERVDVRLDDDGNFQLMNDPGAPWKIWMLRMVCLAISAYTPWAILPSVVGFWITLQYTKRGGVLWDTPSPKEYKKGDTTTGVYRIMTRGLLGSYQAGAGVMVEGVFHTLWHTTKGAALMSGEGRLDPYWGSVKEDRLCYGGPWKLQHKWNGQDEVQMIVVEPGKNVKNVQTKPGVFKTPEGEIGAVTLDFPTGTSGSPIVDKNGDVIGLYGNGVIMPNGSYISAIVQGERMDEPIPAGFEPEMLRKKQITVLDLHPGAGKTRRILPQIIKEAINRRLRTAVLAPTRVVAAEMAEALRGLPIRYQTSAVPREHNGNEIVDVMCHATLTHRLMSPHRVPNYNLFVMDEAHFTDPASIAARGYISTKVELGEAAAIFMTATPPGTSDPFPESNSPISDLQTEIPDRAWNSGYEWITEYTGKTVWFVPSVKMGNEIALCLQRAGKKVVQLNRKSYETEYPKCKNDDWDFVITTDISEMGANFKASRVIDSRKSVKPTIITEGEGRVILGEPSAVTAASAAQRRGRIGRNPSQVGDEYCYGGHTNEDDSNFAHWTEARIMLDNINMPNGLIAQFYQPEREKVYTMDGEYRLRGEERKNFLELLRTADLPVWLAYKVAAAGVSYHDRRWCFDGPRTNTILEDNNEVEVITKLGERKILRPRWIDARVYSDHQALKAFKDFASGKRSQIGLIEVLGKMPEHFMGKTWEALDTMYVVATAEKGGRAHRMALEELPDALQTIALIALLSVMTMGVFFLLMQRKGIGKIGLGGAVLGVATFFCWMAEVPGTKIAGMLLLSLLLMIVLIPEPEKQRSQTDNQLAVFLICVMTLVSAVAANEMGWLDKTKSDISSLFGQRIEVKENFSMGEFLLDLRPATAWSLYAVTTAVLTPLLKHLITSDYINTSLTSINVQASALFTLARGFPFVDVGVSALLLAAGCWGQVTLTVTVTAATLLFCHYAYMVPGWQAEAMRSAQRRTAAGIMKNAVVDGIVATDVPELERTTPIMQKKVGQIMLILVSLAAVVVNPSVKTVREAGILITAAAVTLWENGASSVWNATTAIGLCHIMRGGWLSCLSITWTLIKNMEKPGLKRGGAKGRTLGEVWKERLNQMTKEEFTRYRKEAIIEVDRSAAKHARKEGNVTGGHPVSRGTAKLRWLVERRFLEPVGKVIDLGCGRGGWCYYMATQKRVQEVRGYTKGGPGHEEPQLVQSYGWNIVTMKSGVDVFYRPSECCDTLLCDIGESSSSAEVEEHRTIRVLEMVEDWLHRGPREFCVKVLCPYMPKVIEKMELLQRRYGGGLVRNPLSRNSTHEMYWVSRASGNVVHSVNMTSQVLLGRMEKRTWKGPQYEEDVNLGSGTRAVGKPLLNSDTSKIKNRIERLRREYSSTWHHDENHPYRTWNYHGSYDVKPTGSASSLVNGVVRLLSKPWDTITNVTTMAMTDTTPFGQQRVFKEKVDTKAPEPPEGVKYVLNETTNWLWAFLAREKRPRMCSREEFIRKVNSNAALGAMFEEQNQWRSAREAVEDPKFWEMVDEEREAHLRGECHTCIYNMMGKREKKPGEFGKAKGSRAIWFMWLGARFLEFEALGFLNEDHWLGRKNSGGGVEGLGLQKLGYILREVGTRPGGKIYADDTAGWDTRITRADLENEAKVLELLDGEHRRLARAIIELTYRHKVVKVMRPAADGRTVMDVISREDQRGSGQVVTYALNTFTNLAVQLVRMMEGEGVIGPDDVEKLTKGKGPKVRTWLFENGEERLSRMAVSGDDCVVKPLDDRFATSLHFLNAMSKVRKDIQEWKPSTGWYDWQQVPFCSNHFTELIMKDGRTLVVPCRGQDELVGRARISPGAGWNVRDTACLAKSYAQMWLLLYFHRRDLRLMANAICSAVPVNWVPTGRTTWSIHAGGEWMTTEDMLEVWNRVWIEENEWMEDKTPVEKWSDVPYSGKREDIWCGSLIGTRARATWAENIQVAINQVRAIIGDEKYVDYMSSLKRYEDTTLVEDTVL

SEQ ID NO: 3 - DNA, 8681 bp, Yellow fever virus
agtaaatcctgtgtgctaattgaggtgcattggtctgcaaatcgagttgctaggcaataaacacatttggattaattttaatcgttcgttgagcgattagcagagaactgaccagaacatgtctggtcgtaaagctcagggaaaaaccctgggcgtcaatatggtacgacgaggagttcgctccttgtcaaactcgcgaaacatgacaatgtccatgagcatgatcttggtaggagtgatcatgatgtttttgtctctaggagttggggcggatcaaggatgcgccatcaactttggcaagagagagctcaagtgcggagatggtatcttcatatttagagactctgatgactggctgaacaagtactcatactatccagaagatcctgtgaagcttgcatcaatagtgaaagcctcttttgaagaagggaagtgtggcctaaattcagttgactcccttgagcatgagatgtggagaagcagggcagatgagatcaatgccatttttgaggaaaacgaggtggacatttctgttgtcgtgcaggatccaaagaatgtttaccagagaggaactcatccattttccagaattcgggatggtctgcagtatggttggaagacttggggtaagaaccttgtgttctccccagggaggaagaatggaagcttcatcatagatggaaagtccaggaaagaatgcccgttttcaaaccgggtctggaattctttccagatagaggagtttgggacgggagtgttcaccacacgcgtgtacatggacgcagtctttgaatacaccatagactgcgatggatctatcttgggtgcagcggtgaacggaaaaaagagtgcccatggctctccaacattttggatgggaagtcatgaagtaaatgggacatggatgatccacaccttggaggcattagattacaaggagtgtgagtggccactgacacatacgattggaacatcagttgaagagagtgaaatgttcatgccgagatcaatcggaggcccagttagctctcacaatcatatccctggatacaaggttcagacgaacggaccttggatgcaggtaccactagaagtgaagagagaagcttgcccagggactagcgtgatcattgatggcaactgtgatggacggggaaaatcaaccagatccaccacggatagcgggaaagttattcctgaatggtgttgccgctcctgcacaatgccgcctgtgagcttccatggtagtgatgggtgttggtatcccatggaaattaggccaaggaaaacgcatgaaagccatctggtgcgctcctgggttacagctggagaaatacatgctgtcccttttggtttggtgagcatgatgatagcaatggaagtggtcctaaggaaaagacagggaccaaagcaaatgttggttggaggagtagtgctcttgggagcaatgctggtcgggcaagtaactctccttgatttgctgaaactcacagtggctgtgggattgcatttccatgagatgaacaatggaggagacgccatgtatatggcgttgattgctgccttttcaatcagaccagggctgctcatcggctttgggctcaggaccctatggagccctcgggaacgccttgtgctgaccctaggagcagccatggtggagattgccttgggtggcgtgatgggcggcctgtggaagtatctaaatgcagtttctctctgcatcctgacaataaatgctgttgcttctaggaaagcatcaaataccatcttgcccctcatggctctgttgacacctgtcactatggctgaggtgagacttgccgcaatgttcttttgtgccgtggttatcataggggtccttcaccagaatttcaaggacacctccatgcagaagactatacctctggtggccctcacactcacatcttacctgggcttgacacaaccttttttgggcctgtgtgcatttctggcaacccgcatatttgggcgaaggagtatcccagtgaatgaggcactcgcagcagctggtctagtgggagtgctggcaggactggcttttcaggagatggagaacttccttggtccgattgcagttggaggactcctgatgatgctggttagcgtggctgggagggtggatgggctagagctcaagaagcttggtgaagtttcatgggaagaggaggcggagatcagcgggagttccgcccgctatgatgtggcactcagtgaacaaggggagttcaagctgctttctgaagagaaagtgccatgggaccaggttgtgatgacctcgctggccttggttggggctgccctccatccatttgcacttctgctggtccttgctgggtggctgtttcatgtcaggggagctaggagaagtggggatgtcttgtgggatattcccactcctaagatcatcgaggaatgtgaacatctggaggatgggatttatggcatattccagtcaaccttcttgggggcctcccagcgaggagtgggagtggcacagggaggggtgttccacacaatgtggcatgtcacaagaggagctttccttgtcaggaatggcaagaagttgattccatcttgggcttcagtaaaggaagaccttgtcgcctatggtggctcatggaagttggaaggcagatgggatggagaggaagaggtccagttgatcgcggctgttccaggaaagaacgtggtcaacgtccagacaaaaccgagcttgttcaaagtgaggaatgggggagaaatcggggctgtcgctcttgactatccgagtggcacttcaggatctcctattgttaacaggaacggagaggtgattgggctgtacggcaatggcatccttgtcggtgacaactccttcgtgtccgccatatcccagactgaggtgaaggaagaaggaaaggaggagctccaagagatcccgacaatgctaaagaaaggaatgacaactgtccttgattttcatcctggagctgggaagacaagacgtttcctcccacagatcttggccgagtgcgcacggagacgcttgcgcactcttgtgttggcccccaccagggttgttctttctgaaatgaaggaggcttttcacggcctggacgtgaaattccacacacaggctttttccgctcacggcagcgggagagaagtcattgatgccatgtgccatgccaccctaacttacaggatgttggaaccaactagggttgttaactgggaagtgatcattatggatgaagcccattttttggatccagctagcatagccgctagaggttgggcagcgcacagagctagggcaaatgaaagtgcaacaatcttgatgacagccacaccgcctgggactagtgatgaatttccacattcaaatggtgaaatagaagatgttcaaacggacatacccagtgagccctggaacacagggcatgactggatcctagctgacaaaaggcccacggcatggttccttccatccatcagagctgcaaatgtcatggctgcctctttgcgtaaggctggaaagagtgtggtggtcctgaacaggaaaacctttgagagagaataccccacgataaagcagaagaaacctgactttatattggccactgacatagctgaaatgggagccaacctttgcgtggagcgagtgctggattgcaggacggcttttaagcctgtgcttgtggatgaagggaggaaggtggcaataaaagggccacttcgtatctccgcatcctctgctgctcaaaggagggggcgcattgggagaaatcccaacagagatggagactcatactactattctgagcctacaagtgaaaataatgcccaccacgtctgctggttggaggcctcaatgctcttggacaacatggaggtgaggggtggaatggtcgccccactctatggcgttgaaggaactaaaacaccagtttcccctggtgaaatgagactgagggatgaccagaggaaagtcttcagagaactagtgaggaattgtgacctgcccgtttggctttcgtggcaagtggccaaggctggtttgaagacgaatgatcgtaagtggtgttttgaaggccctgaggaacatgagatcttgaatgacagcggtgaaacagtgaagtgcagggctcctggaggagcaaagaagcctctgcgcccaaggtggtgtgatgaaagggtgtcatctgaccagagtgcgctgtctgaatttattaagtttgctgaaggtaggaggggagctgctgaagtgctagttgtgctgagtgaactccctgatttcctggctaaaaaaggtggagaggcaatggataccatcagtgtgtttctccactctgaggaaggctctagggcttaccgcaatgcactatcaatgatgcctgaggcaatgacaatagtcatgctgtttatactggctggactactgacatcgggaatggtcatctttttcatgtctcccaaaggcatcagtagaatgtctatggcgatgggcacaatggccggctgtggatatctcatgttccttggaggcgtcaaacccactcacatctcctatatcatgctcatattctttgtcctgatggtggttgtgatccccgagccagggcaacaaaggtccatccaagacaaccaagtggcatacctcattattggcatcctgacgctggtttcagcggtggcagccaacgagctaggcatgctggagaaaaccaaagaggacctctttgggaagaagaacttaattccatctagtgcttcaccctggagttggccggatcttgacctgaagccaggagctgcctggacagtgtacgttggcattgttacaatgctctctccaatgttgcaccactggatcaaagtcgaatatggcaacctgtctctgtctggaatagcccagtcagcctcagtcctttctttcatggacaaggggataccattcatgaagatgaatatctcggtcataatgctgctggtcagtggctggaattcaataacagtgatgcctctgctctgtggcatagggtgcgccatgctccactggtctctcattttacctggaatcaaagcgcagcagtcaaagcttgcacagagaagggtgttccatggcgttgccaagaaccctgtggttgatgggaatccaacagttgacattgaggaagctcctgaaatgcctgccctttatgagaagaaactggctctatatctccttcttgctctcagcctagcttctgttgccatgtgcagaacgcccttttcattggctgaaggcattgtcctagcatcagctgccttagggccgctcatagagggaaacaccagccttctttggaatggacccatggctgtctccatgacaggagtcatgagggggaatcactatgcttttgtgggagtcatgtacaatctatggaagatgaaaactggacgccgggggagcgcgaatggaaaaactttgggtgaagtctggaagagggaactgaatctgttggacaagcgacagtttgagttgtataaaaggaccgacattgtggaggtggatcgtgatacggcacgcaggcatttggccgaagggaaggtggacaccggggtggcggtctccagggggaccgcaaagttaaggtggttccatgagcgtggctatgtcaagctggaaggtagggtgattgacctggggtgtggccgcggaggctggtgttactacgctgctgcgcaaaaggaagtgagtggggtcaaaggatttactcttggaagagacggccatgagaaacccatgaatgtgcaaagtctgggatggaacatcatcaccttcaaggacaaaactgatatccaccgcctagaaccagtgaaatgtgacacccttttgtgtgacattggagagtcatcatcgtcatcggtcacagagggggaaaggaccgtgagagttcttgatactgtagaaaaatggctggcttgtggggttgacaacttctgtgtgaaggtgttagctccatacatgccagatgttctcgagaaactggaattgctccaaaggaggtttggcggaacagtgatcaggaaccctctctccaggaattccactcatgaaatgtactacgtgtctggagcccgcagcaatgtcacatttactgtgaaccaaacatcccgcctcctgatgaggagaatgaggcgtccaactggaaaagtgaccctggaggctgacgtcatcctcccaattgggacacgcagtgttgagacagacaagggacccctggacaaagaggccatagaagaaagggttgagaggataaaatctgagtacatgacctcttggttttatgacaatgacaacccctacaggacctggcactactgtggctcctatgtcacaaaaacctcaggaagtgcggcgagcatggtaaatggtgttattaaaattctgacatatccatgggacaggatagaggaggtcacaagaatggcaatgactgacacaaccccttttggacagcaaagagtgtttaaagaaaaagttgacaccagagcaaaggatccaccagcgggaactaggaagatcatgaaagttgtcaacaggtggctgttccgccacctggccagagaaaagaaccccagactgtgcacaaaggaagaatttattgcaaaagtccgaagtcatgcagccattggagcttacctggaagaacaagaacagtggaagactgccaatgaggctgtccaagacccaaagttctgggaactggtggatgaagaaaggaagctgcaccaacaaggcaggtgtcggacttgtgtgtacaacatgatggggaaaagagagaagaagctgtcagagtttgggaaagcaaagggaagccgtgccatatggtatatgtggctgggagcgcggtatcttgagtttgaggccctgggattcctgaatgaggaccattgggcttccagggaaaactcaggaggaggagtggaaggcattggcttacaatacctaggatatgtgatcagagacctggctgcaatggatggtggtggattctacgcggatgacaccgctggatgggacacgcgcatcacagaggcagaccttgatgatgaacaggagatcttgaactacatgagcccacatcacaaaaaactggcacaagcagtgatggaaatgacatacaagaacaaagtggtgaaagtgttgagaccagccccaggagggaaagcctacatggatgtcataagtcgacgagaccagagaggatccgggcaggtagtgacttatgctctgaacaccatcaccaacttgaaagtccaattgatcagaatggcagaagcagagatggtgatacatcaccaacatgttcaagattgtgatgaatcagttctgaccaggctggaggcatggctcactgagcacggatgtaacagactgaagaggatggcggtgagtggagacgactgtgtggtccggcccatcgatgacaggttcggcctggccctgtcccatctcaacgccatgtccaaggttagaaaggacatatctgaatggcagccatcaaaagggtggaatgattgggagaatgtgcccttctgttcccaccacttccatgaactacagctgaaggatggcaggaggattgtggtgccttgccgagaacaggacgagctcattgggagaggaagggtgtctccaggaaacggctggatgatcaaggaaacagcttgcctcagcaaagcctatgccaacatgtggtcactgatgtattttcacaaaagggacatgaggctactgtcattggctgtttcctcagctgttcccacctcatgggttccacaaggacgcacaacatggtcgattcatgggaaaggggagtggatgaccacggaagacatgcttgaggtgtggaacagagtatggataaccaacaacccacacatgcaggacaagacaatggtgaaaaaatggagagatgtcccttatctaaccaagagacaagacaagctgtgcggatcactgattggaatgaccaatagggccacctgggcctcccacatccatttagtcatccatcgtatccgaacgctgattggacaggagaaatacactgactacctaacagtcatggacaggtattctgtggatgctgacctgcaactgggtgagcttatctgaaacaccatctaacaggaataaccgggatacaaaccacgggtggagaaccggactccccacaacctgaaaccgggatataaaccacggctggagaaccggactccgcacttaaaatgaaacagaaaccgggataaaaactacggatggagaaccggactccacacattgagacagaagaagttgtcagcccagaaccccacacgagttttgccactgctaagctgtgaggcagtgcaggctgggacagccgacctccaggttgcgaaaaacctggtttctgggacctcccaccccagagtaaaaagaacggagcctccgctaccaccctcccacgtggtggtagaaagacggggtctagaggttagagaagaccctccagggaacaaatagtgggaccatattgacgccagggaaagaccggagtggttctctgcttttcctccagaggtctgtgagcacagtttgctcaagaataagcagacctttggatgacaaacacaaaaccact

SEQ ID NO: 4 - protein, 2684 aa, Yellow fever virus
MSGRKAQGKTLGVNMVRRGVRSLSNSRNMTMSMSMILVGVIMMFLSLGVGADQGCAINFGKRELKCGDGIFIFRDSDDWLNKYSYYPEDPVKLASIVKASFEEGKCGLNSVDSLEHEMWRSRADEINAIFEENEVDISVVVQDPKNVYQRGTHPFSRIRDGLQYGWKTWGKNLVFSPGRKNGSFIIDGKSRKECPFSNRVWNSFQIEEFGTGVFTTRVYMDAVFEYTIDCDGSILGAAVNGKKSAHGSPTFWMGSHEVNGTWMIHTLEALDYKECEWPLTHTIGTSVEESEMFMPRSIGGPVSSHNHIPGYKVQTNGPWMQVPLEVKREACPGTSVIIDGNCDGRGKSTRSTTDSGKVIPEWCCRSCTMPPVSFHGSDGCWYPMEIRPRKTHESHLVRSWVTAGEIHAVPFGLVSMMIAMEVVLRKRQGPKQMLVGGVVLLGAMLVGQVTLLDLLKLTVAVGLHFHEMNNGGDAMYMALIAAFSIRPGLLIGFGLRTLWSPRERLVLTLGAAMVEIALGGVMGGLWKYLNAVSLCILTINAVASRKASNTILPLMALLTPVTMAEVRLAAMFFCAVVIIGVLHQNFKDTSMQKTIPLVALTLTSYLGLTQPFLGLCAFLATRIFGRRSIPVNEALAAAGLVGVLAGLAFQEMENFLGPIAVGGLLMMLVSVAGRVDGLELKKLGEVSWEEEAEISGSSARYDVALSEQGEFKLLSEEKVPWDQVVMTSLALVGAALHPFALLLVLAGWLFHVRGARRSGDVLWDIPTPKIIEECEHLEDGIYGIFQSTFLGASQRGVGVAQGGVFHTMWHVTRGAFLVRNGKKLIPSWASVKEDLVAYGGSWKLEGRWDGEEEVQLIAAVPGKNVVNVQTKPSLFKVRNGGEIGAVALDYPSGTSGSPIVNRNGEVIGLYGNGILVGDNSFVSAISQTEVKEEGKEELQEIPTMLKKGMTTVLDFHPGAGKTRRFLPQILAECARRRLRTLVLAPTRVVLSEMKEAFHGLDVKFHTQAFSAHGSGREVIDAMCHATLTYRMLEPTRVVNWEVIIMDEAHFLDPASIAARGWAAHRARANESATILMTATPPGTSDEFPHSNGEIEDVQTDIPSEPWNTGHDWILADKRPTAWFLPSIRAANVMAASLRKAGKSVVVLNRKTFEREYPTIKQKKPDFILATDIAEMGANLCVERVLDCRTAFKPVLVDEGRKVAIKGPLRISASSAAQRRGRIGRNPNRDGDSYYYSEPTSENNAHHVCWLEASMLLDNMEVRGGMVAPLYGVEGTKTPVSPGEMRLRDDQRKVFRELVRNCDLPVWLSWQVAKAGLKTNDRKWCFEGPEEHEILNDSGETVKCRAPGGAKKPLRPRWCDERVSSDQSALSEFIKFAEGRRGAAEVLVVLSELPDFLAKKGGEAMDTISVFLHSEEGSRAYRNALSMMPEAMTIVMLFILAGLLTSGMVIFFMSPKGISRMSMAMGTMAGCGYLMFLGGVKPTHISYIMLIFFVLMVVVIPEPGQQRSIQDNQVAYLIIGILTLVSAVAANELGMLEKTKEDLFGKKNLIPSSASPWSWPDLDLKPGAAWTVYVGIVTMLSPMLHHWIKVEYGNLSLSGIAQSASVLSFMDKGIPFMKMNISVIMLLVSGWNSITVMPLLCGIGCAMLHWSLILPGIKAQQSKLAQRRVFHGVAKNPVVDGNPTVDIEEAPEMPALYEKKLALYLLLALSLASVAMCRTPFSLAEGIVLASAALGPLIEGNTSLLWNGPMAVSMTGVMRGNHYAFVGVMYNLWKMKTGRRGSANGKTLGEVWKRELNLLDKRQFELYKRTDIVEVDRDTARRHLAEGKVDTGVAVSRGTAKLRWFHERGYVKLEGRVIDLGCGRGGWCYYAAAQKEVSGVKGFTLGRDGHEKPMNVQSLGWNIITFKDKTDIHRLEPVKCDTLLCDIGESSSSSVTEGERTVRVLDTVEKWLACGVDNFCVKVLAPYMPDVLEKLELLQRRFGGTVIRNPLSRNSTHEMYYVSGARSNVTFTVNQTSRLLMRRMRRPTGKVTLEADVILPIGTRSVETDKGPLDKEAIEERVERIKSEYMTSWFYDNDNPYRTWHYCGSYVTKTSGSAASMVNGVIKILTYPWDRIEEVTRMAMTDTTPFGQQRVFKEKVDTRAKDPPAGTRKIMKVVNRWLFRHLAREKNPRLCTKEEFIAKVRSHAAIGAYLEEQEQWKTANEAVQDPKFWELVDEERKLHQQGRCRTCVYNMMGKREKKLSEFGKAKGSRAIWYMWLGARYLEFEALGFLNEDHWASRENSGGGVEGIGLQYLGYVIRDLAAMDGGGFYADDTAGWDTRITEADLDDEQEILNYMSPHHKKLAQAVMEMTYKNKVVKVLRPAPGGKAYMDVISRRDQRGSGQVVTYALNTITNLKVQLIRMAEAEMVIHHQHVQDCDESVLTRLEAWLTEHGCNRLKRMAVSGDDCVVRPIDDRFGLALSHLNAMSKVRKDISEWQPSKGWNDWENVPFCSHHFHELQLKDGRRIVVPCREQDELIGRGRVSPGNGWMIKETACLSKAYANMWSLMYFHKRDMRLLSLAVSSAVPTSWVPQGRTTWSIHGKGEWMTTEDMLEVWNRVWITNNPHMQDKTMVKKWRDVPYLTKRQDKLCGSLIGMTNRATWASHIHLVIHRIRTLIGQEKYTDYLTVMDRYSVDADLQLGELI

SEQ ID NO: 5 - protein, 22 aa, Unknown
  source: /note="Description of Unknown: 2A peptide sequence"
GSGATNFSLLKQAGDVEENPGP

SEQ ID NO: 6 - protein, 33 aa, Unknown
  source: /note="Description of Unknown: 2A peptide sequence"
FARHKQKIVAPVKQTLNFDLLKLAGDVESNPGP

SEQ ID NO: 7 - protein, 25 aa, Unknown
  source: /note="Description of Unknown: 2A peptide sequence"
GSGVKQTLNFDLLKLAGDVESNPGP

SEQ ID NO: 8 - protein, 23 aa, Unknown
  source: /note="Description of Unknown: 2A peptide sequence"
GSGQCTNYALLKLAGDVESNPGP

SEQ ID NO: 9 - protein, 21 aa, Unknown
  source: /note="Description of Unknown: 2A peptide sequence"
GSGEGRGSLLTCGDVEENPGP

SEQ ID NO: 10 - DNA, 576 bp, Encephalomyocarditis virus
cccccccctaacgttactggccgaagccgcttggaataaggccggtgtgcgtttgtctatatgttattttccaccatattgccgtcttttggcaatgtgagggcccggaaacctggccctgtcttcttgacgagcattcctaggggtctttcccctctcgccaaaggaatgcaaggtctgttgaatgtcgtgaaggaagcagttcctctggaagcttcttgaagacaaacaacgtctgtagcgaccctttgcaggcagcggaaccccccacctggcgacaggtgcctctgcggccaaaagccacgtgtataagatacacctgcaaaggcggcacaaccccagtgccacgttgtgagttggatagttgtggaaagagtcaaatggctctcctcaagcgtattcaacaaggggctgaaggatgcccagaaggtaccccattgtatgggatctgatctggggcctcggtgcacatgctttacatgtgtttagtcgaggttaaaaaacgtctaggccccccgaaccacggggacgtggttttcctttgaaaaacacgatgataatatggccacaaccatg

SEQ ID NO: 11 - DNA, 746 bp, Encephalomyocarditis virus
ttaaaacagctgtgggttgttcccacccacagggcccactgggcgctagcactctgattttacgaaatccttgtgcgcctgttttatatcccttccctaattcgaaacgtagaagcaatgcgcaccactgatcaatagtaggcgtaacgcgccagttacgtcatgatcaagcatatctgttcccccggactgagtatcaatagactgcttacgcggttgaaggagaaaacgttcgttatccggctaactacttcgagaagcccagtaacaccatggaagctgcagggtgtttcgctcagcacttcccccgtgtagatcaggtcgatgagccactgcaatccccacaggtgactgtggcagtggctgcgttggcggcctgcctatggggagacccataggacgctctaatgtggacatggtgcgaagagcctattgagctagttagtagtcctccggcccctgaatgcggctaatcctaactgcggagcacatgccttcaacccagagggtagtgtgtcgtaatgggcaactctgcagcggaaccgactactttgggtgtccgtgtttctttttattcttatattggctgcttatggtgacaattacagaattgttaccatatagctattggattggccatccggtgtgtaatagagctgttatatacctatttgttggctttgtaccactaactttaaaatctataactaccctcaactttatattaaccctcaatacagttgaac

SEQ ID NO: 12 - DNA, 360 bp, Hepatitis C virus
gccagcccccgattgggggcgacactccaccatagatcactcccctgtgaggaactactgtcttcacgcagaaagcgtctagccatggcgttagtatgagtgtcgtgcagcctccaggcccccccctcccgggagagccatagtggtctgcggaaccggtgagtacaccggaattgccaggacgaccgggtcctttcttggatcaatcccgctcaatgcctggagatttgggcgtgcccccgcgagactgctagccgagtagtgttgggtcgcgaaaggccttgtggtactgcctgatagggtgcttgcgagtgccccgggaggtctcgtagaccgtgcaccatgagcacgaatcctaaa

SEQ ID NO: 13 - DNA, 211 bp, Cricket paralysis virus
ctaaaaagcaaaaatgtgatcttgcttgtaaatacaattttgagaggttaataaattacaagtagtgctatttttgtatttaggttagctatttagctttacgttccaggatgcctagtggcagccccacaatatccaggaagccctctctgcggtttttcagattaggtagtcgaaaaacctaagaaatttacctgctacatttcaagat

SEQ ID NO: 14 - DNA, 618 bp, Human rhinovirus
ttaaaactgggagtgggttgttcccactcactccacccatgcggtgttgtactctgttattacggtaactttgtacgccagtttttcccacccttccccataatgtaacttagaagtttgtacaatatgaccaataggtgacaatcatccagactgtcaaaggtcaagcacttctgtttccccggtcaatgaggatatgctttacccaaggcaaaaaccttagagatcgttatccccacactgcctacacagagcccagtaccatttttgatataattgggttggtcgctccctgcaaacccagcagtagacctggcagatgaggctggacattccccactggcgacagtggtccagcctgcgtggctgcctgctcacccttcttgggtgagaagcctaattattgacaaggtgtgaagagccgcgtgtgctcagtgtgcttcctccggcccctgaatgtggctaaccttaaccctgcagccgttgcccataatccaatgggtttgcggtcgtaatgcgtaagtgcgggatgggaccaactactttgggtgtccgtgtttcctgtttttcttttgattgcattttatggtgacaatttatagtgtatagattgtcatc

SEQ ID NO: 15 - DNA, 741 bp, Coxsackievirus
ttaaaacagcctgtgggttgttcccacccacaggcccattgggcgctagcactctggtatcacggtacctttgtgcgcctgttttacatcccctccccaaattgtaatttagaagtttcacacaccgatcattagcaagcgtggcacaccagccatgttttgatcaagcacttctgttaccccggactgagtatcaatagaccgctaacgcggttgaaggagaaaacgttcgttacccggccaactacttcgaaaaacctagtaacaccatggaagttgcggagtgtttcgctcagcactaccccagtgtagatcaggtcgatgagtcaccgcgttccccacgggcgaccgtggcggtggctgcgttggcggcctgcctacggggaaacccgtaggacgctctaatacagacatggtgcgaagagtctattgagctagttggtaatcctccggcccctgaatgcggctaatcctaactgcggagcacataccctcaaaccagggggcagtgtgtcgtaacgggcaactctgcagcggaaccgactactttgggtgtccgtgtttcattttattcctatactggctgcttatggtgacaattgacaggttgttaccatatagttattggattggccatccggtgactaacagagcaattatatatctctttgttgggtttataccacttagcttgaaagaggttaaaacactacatctcatcattaaactaaatacaacaaa

SEQ ID NO: 16 - DNA, 279 bp, West Nile virus
agtagttcgcctgtgtgagctgacaaacttagtagtgtttgtgaggattaacaacaattaacacagtgcgagctgtttcttagcacgaagatctcgatgtctaagaaaccaggagggcccggcaagagccgggctgtcaatatgctaaaacgcggaatgccccgcgtgttgtccttgattggacttaagatgggcatcaatgctcgtgataggtccatagctctcacgtttctcgcagttggaggagttctgctcttcctctccgtgaacgtgcacgct

SEQ ID NO: 17 - DNA, 271 bp, Yellow fever virus
agtaaatcctgtgtgctaattgaggtgcattggtctgcaaatcgagttgctaggcaataaacacatttggattaattttaatcgttcgttgagcgattagcagagaactgaccagaacatgtctggtcgtaaagctcagggaaaaaccctgggcgtcaatatggtacgacgaggagttcgctccttgtcaaactcgcgaaacatgacaatgtccatgagcatgatcttggtaggagtgatcatgatgtttttgtctctaggagttggggcg

SEQ ID NO: 18 - DNA, 90 bp, West Nile virus
atgggcatcaatgctcgtgataggtccatagctctcacgtttctcgcagttggaggagttctgctcttcctctccgtgaacgtgcacgct

SEQ ID NO: 19 - protein, 30 aa, West Nile virus
MGINARDRSIALTFLAVGGVLLFLSVNVHA

SEQ ID NO: 20 - DNA, 74 bp, Yellow fever virus
gaaacatgacaatgtccatgagcatgatcttggtaggagtgatcatgatgtttttgtctctaggagttggggcg

SEQ ID NO: 21 - protein, 24 aa, Yellow fever virus
NMTMSMSMILVGVIMMFLSLGVGA

SEQ ID NO: 22 - DNA, 19 bp, Artificial Sequence
  source: /note="Description of Artificial Sequence: Synthetic oligonucleotide"
taatacgactcactataga

SEQ ID NO: 23 - DNA, 19 bp, Artificial Sequence
  source: /note="Description of Artificial Sequence: Synthetic oligonucleotide"
taatacgactcactattaa

SEQ ID NO: 24 - DNA, 19 bp, Artificial Sequence
  source: /note="Description of Artificial Sequence: Synthetic oligonucleotide"
taatacgactcactataaa

SEQ ID NO: 25 - DNA, 18 bp, Artificial Sequence
  source: /note="Description of Artificial Sequence: Synthetic oligonucleotide"
taatacgactcactatta

SEQ ID NO: 26 - DNA, 18 bp, Artificial Sequence
  source: /note="Description of Artificial Sequence: Synthetic oligonucleotide"
taatacgactcactataa

SEQ ID NO: 27 - DNA, 11 bp, Artificial Sequence
  source: /note="Description of Artificial Sequence: Synthetic oligonucleotide"
gatctctagat